European Patent Application EP 4 410 841 A1, published August 7, 2024. Title: ANTI-IL23 ANTIBODY FUSION PROTEIN AND USES THEREOF. Applicant: JIANGSU HENGRUI PHARMACEUTICALS CO., LTD. Application CN PCT/CN2022/123370, filed September 30, 2022. The sequence listing filed with the application follows.

SEQUENCE LISTING (85 sequences)

SEQ ID NO: 1 - protein, 121 aa, Mus musculus
  DOMAIN 1..121: note = mAb29
QVQLKESGPGLVAPSQSLSITCTVSGFSLTSYAISWVRQPPGKGLEWLGVIWTGGGTNYNSGIKSRLTISKDNSKSQVFLNMNSLQTEDTARYYCVREGDYGSYAGAMDYWGQGTSVTVSS

SEQ ID NO: 2 - protein, 111 aa, Mus musculus
  DOMAIN 1..111: note = mAb29
DIVLTQSPASLAVSLGQRATISCRASESVDYYGISSMHWFQQKPGQPPKLLIYRASNLESGIPARFSGSGSRTDFTLTINRVETDDVATYYCQQANKDPYTFGGGTKLEIK

SEQ ID NO: 3 - protein, 114 aa, Mus musculus
  DOMAIN 1..114: note = mAb38
EFQLQQSGPELVKPGASVKISCKASGYSFTDHNMNWVKQSNGKSLEWIGVINPNYGTTTYNQKFKGKATLTVDQSSSTAYMQLNILTSEDSAVYYCARRGFAYWGQGTLVTVSA

SEQ ID NO: 4 - protein, 112 aa, Mus musculus
  DOMAIN 1..112: note = mAb38
DIVISQDELSNPVTSGESVSISCRSSKSLLYKDGKTYLNWFLQRPGQSPQLLIYLMSTRASGVSDRFSGSGSGTDLTLEISRVKAEDVGVYYCQQIAEYPFTFGSGTKLEIK

SEQ ID NO: 5 - protein, 5 aa, synthetic construct
  DOMAIN 1..5: note = mAb29HCDR1
SYAIS

SEQ ID NO: 6 - protein, 16 aa, synthetic construct
  DOMAIN 1..16: note = mAb29HCDR2
VIWTGGGTNYNSGIKS

SEQ ID NO: 7 - protein, 13 aa, synthetic construct
  DOMAIN 1..13: note = mAb29HCDR3
EGDYGSYAGAMDY

SEQ ID NO: 8 - protein, 15 aa, synthetic construct
  DOMAIN 1..15: note = mAb29LCDR1
RASESVDYYGISSMH

SEQ ID NO: 9 - protein, 7 aa, synthetic construct
  DOMAIN 1..7: note = mAb29LCDR2
RASNLES

SEQ ID NO: 10 - protein, 9 aa, synthetic construct
  DOMAIN 1..9: note = mAb29LCDR3
QQANKDPYT

SEQ ID NO: 11 - protein, 5 aa, synthetic construct
  DOMAIN 1..5: note = mAb38HCDR1
DHNMN

SEQ ID NO: 12 - protein, 17 aa, synthetic construct
  DOMAIN 1..17: note = mAb38HCDR2
VINPNYGTTTYNQKFKG

SEQ ID NO: 13 - protein, 5 aa, synthetic construct
  DOMAIN 1..5: note = mAb38HCDR3
RGFAY

SEQ ID NO: 14 - protein, 16 aa, synthetic construct
  DOMAIN 1..16: note = mAb38LCDR1
RSSKSLLYKDGKTYLN

SEQ ID NO: 15 - protein, 7 aa, synthetic construct
  DOMAIN 1..7: note = mAb38LCDR2
LMSTRAS

SEQ ID NO: 16 - protein, 9 aa, synthetic construct
  DOMAIN 1..9: note = mAb38LCDR3
QQIAEYPFT

SEQ ID NO: 17 - protein, 121 aa, synthetic construct
  DOMAIN 1..121: note = hAb29VH1
EVTLKESGPVLVKPTETLTLTCTVSGFSLSSYAISWIRQPPGKALEWLGVIWTGGGTNYNSGIKSRLTISKDTSKSQVVLTMTNMDPVDTATYYCVREGDYGSYAGAMDYWGQGTTVTVSS

SEQ ID NO: 18 - protein, 121 aa, synthetic construct
  DOMAIN 1..121: note = hAb29VH2
EVTLKESGPVLVKPTETLTLTCTVSGFSLTSYAISWIRQPPGKALEWLGVIWTGGGTNYNSGIKSRLTISKDNSKSQVVLTMTNMDPVDTATYYCVREGDYGSYAGAMDYWGQGTTVTVSS

SEQ ID NO: 19 - protein, 121 aa, synthetic construct
  DOMAIN 1..121: note = hAb29VH3
EVTLKESGPVLVKPTETLTLTCTVSGFSLTSYAISWVRQPPGKALEWLGVIWTGGGTNYNSGIKSRLTISKDNSKSQVVLTMTNMDPVDTARYYCVREGDYGSYAGAMDYWGQGTTVTVSS

SEQ ID NO: 20 - protein, 121 aa, synthetic construct
  DOMAIN 1..121: note = hAb29VH4
QVTLKESGPVLVKPTETLTLTCTVSGFSLTSYAISWVRQPPGKGLEWLGVIWTGGGTNYNSGIKSRLTISKDNSKSQVVLTMTNMDPVDTARYYCVREGDYGSYAGAMDYWGQGTTVTVSS

SEQ ID NO: 21 - protein, 121 aa, synthetic construct
  DOMAIN 1..121: note = hAb29VH5
QVTLKESGPVLVKPTETLTLTCTVSGFSLTNYAISWVRQPPGKGLEWLGVIWTGGGTNYNSGIKSRLTISKDNSKSQVVLTMTNMDPVDTARYYCVREGDYGSYAGAMDYWGQGTTVTVSS

SEQ ID NO: 22 - protein, 121 aa, synthetic construct
  DOMAIN 1..121: note = hAb29VH6
QVTLKESGPVLVKPTETLTLTCTVSGFSLTQYAISWVRQPPGKGLEWLGVIWTGGGTNYNSGIKSRLTISKDNSKSQVVLTMTNMDPVDTARYYCVREGDYGSYAGAMDYWGQGTTVTVSS

SEQ ID NO: 23 - protein, 111 aa, synthetic construct
  DOMAIN 1..111: note = hAb29VL1
DIVMTQSPDSLAVSLGERATINCRASESVDYYGISSMHWFQQKPGQPPKLLIYRASNLESGVPDRFSGSGSRTDFTLTISSLQAEDVAVYYCQQANKDPYTFGGGTKVEIK

SEQ ID NO: 24 - protein, 111 aa, synthetic construct
  DOMAIN 1..111: note = hAb29VL2
DIVLTQSPDSLAVSLGERATINCRASESVDYYGISSMHWFQQKPGQPPKLLIYRASNLESGIPDRFSGSGSRTDFTLTISSLQAEDVAVYYCQQANKDPYTFGGGTKVEIK

SEQ ID NO: 25 - protein, 111 aa, synthetic construct
  DOMAIN 1..111: note = hAb29VL3
DIVLTQSPDSLAVSLGERATINCRASESVDYYGISSMHWFQQKPGQPPKLLIYRASNLESGIPARFSGSGSRTDFTLTISSLQAEDVAVYYCQQANKDPYTFGGGTKVEIK

SEQ ID NO: 26 - protein, 111 aa, synthetic construct
  DOMAIN 1..111: note = hAb29VL4
DIVLTQSPDSLAVSLGQRATINCRASESVDYYGISSMHWFQQKPGQPPKLLIYRASNLESGIPARFSGSGSRTDFTLTISSLQAEDVAVYYCQQANKDPYTFGGGTKVEIK

SEQ ID NO: 27 - protein, 5 aa, synthetic construct
  DOMAIN 1..5: note = hAb29VH5HCDR1
NYAIS

SEQ ID NO: 28 - protein, 5 aa, synthetic construct
  DOMAIN 1..5: note = hAb29VH6HCDR1
QYAIS

SEQ ID NO: 29 - protein, 114 aa, synthetic construct
  DOMAIN 1..114: note = hAb38VH1
EFQLVQSGAEVKKPGASVKVSCKASGYTFTDHNMNWVRQAPGQRLEWMGVINPNYGTTTYNQKFKGRVTITVDTSASTAYMELSSLRSEDTAVYYCARRGFAYWGQGTLVTVSS

SEQ ID NO: 30 - protein, 114 aa, synthetic construct
  DOMAIN 1..114: note = hAb38VH2
EVQLVQSGAEVKKPGASVKVSCKASGYSFTDHNMNWVRQAPGQRLEWMGVINPNYGTTTYNQKFKGRVTITVDTSASTAYMELSSLRSEDTAVYYCARRGFAYWGQGTLVTVSS

SEQ ID NO: 31 - protein, 114 aa, synthetic construct
  DOMAIN 1..114: note = hAb38VH3
EFQLVQSGAEVKKPGASVKVSCKASGYSFTDHNMNWVRQAPGQRLEWMGVINPNYGTTTYNQKFKGRVTITVDQSASTAYMELSSLRSEDTAVYYCARRGFAYWGQGTLVTVSS

SEQ ID NO: 32 - protein, 114 aa, synthetic construct
  DOMAIN 1..114: note = hAb38VH4
EFQLVQSGAEVKKPGASVKVSCKASGYSFTDHNMNWVRQAPGQSLEWMGVINPNYGTTTYNQKFKGRVTITVDQSASTAYMELSSLRSEDTAVYYCARRGFAYWGQGTLVTVSS

SEQ ID NO: 33 - protein, 112 aa, synthetic construct
  DOMAIN 1..112: note = hAb38VL1
DIVMTQTPLSLPVTPGEPASISCRSSKSLLYKDGKTYLNWYLQKPGQSPQLLIYLMSTRASGVPDRFSGSGSGTDFTLKISRVEAEDVGVYYCQQIAEYPFTFGSGTKLEIK

SEQ ID NO: 34 - protein, 112 aa, synthetic construct
  DOMAIN 1..112: note = hAb38VL2
DIVMTQTPLSLPVTPGEPASISCRSSKSLLYKDGKTYLNWFLQKPGQSPQLLIYLMSTRASGVPDRFSGSGSGTDLTLKISRVEAEDVGVYYCQQIAEYPFTFGSGTKLEIK

SEQ ID NO: 35 - protein, 112 aa, synthetic construct
  DOMAIN 1..112: note = hAb38VL3
DIVITQTPLSLPVTPGEPASISCRSSKSLLYKDGKTYLNWFLQRPGQSPQLLIYLMSTRASGVPDRFSGSGSGTDLTLKISRVEAEDVGVYYCQQIAEYPFTFGSGTKLEIK

SEQ ID NO: 36 - protein, 112 aa, synthetic construct
  DOMAIN 1..112: note = hAb38VL4
DIVMTQTPLSLPVTPGEPASISCRSSKSLLYKDGKTYLNWFLQKPGQSPQLLIYLMQTRASGVPDRFSGSGSGTDLTLKISRVEAEDVGVYYCQQIAEYPFTFGSGTKLEIK

SEQ ID NO: 37 - protein, 7 aa, synthetic construct
  DOMAIN 1..7: note = hAb38VL4LCDR2
LMQTRAS

SEQ ID NO: 38 - protein, 330 aa, synthetic construct
  DOMAIN 1..330: note = IgG1L234AL235A
ASTKGPSVFPLAPSSKSTSGGTAALGCLVKDYFPEPVTVSWNSGALTSGVHTFPAVLQSSGLYSLSSVVTVPSSSLGTQTYICNVNHKPSNTKVDKKVEPKSCDKTHTCPPCPAPEAAGGPSVFLFPPKPKDTLMISRTPEVTCVVVDVSHEDPEVKFNWYVDGVEVHNAKTKPREEQYNSTYRVVSVLTVLHQDWLNGKEYKCKVSNKALPAPIEKTISKAKGQPREPQVYTLPPSRDELTKNQVSLTCLVKGFYPSDIAVEWESNGQPENNYKTTPPVLDSDGSFFLYSKLTVDKSRWQQGNVFSCSVMHEALHNHYTQKSLSLSPGK

SEQ ID NO: 39 - protein, 107 aa, synthetic construct [sequence omitted]

SEQ ID NO: 40 - protein, 451 aa, synthetic construct
  CHAIN 1..451: note = Hu29-19
QVTLKESGPVLVKPTETLTLTCTVSGFSLTNYAISWVRQPPGKGLEWLGVIWTGGGTNYNSGIKSRLTISKDNSKSQVVLTMTNMDPVDTARYYCVREGDYGSYAGAMDYWGQGTTVTVSSASTKGPSVFPLAPSSKSTSGGTAALGCLVKDYFPEPVTVSWNSGALTSGVHTFPAVLQSSGLYSLSSVVTVPSSSLGTQTYICNVNHKPSNTKVDKKVEPKSCDKTHTCPPCPAPEAAGGPSVFLFPPKPKDTLMISRTPEVTCVVVDVSHEDPEVKFNWYVDGVEVHNAKTKPREEQYNSTYRVVSVLTVLHQDWLNGKEYKCKVSNKALPAPIEKTISKAKGQPREPQVYTLPPSRDELTKNQVSLTCLVKGFYPSDIAVEWESNGQPENNYKTTPPVLDSDGSFFLYSKLTVDKSRWQQGNVFSCSVMHEALHNHYTQKSLSLSPGK

SEQ ID NO: 41 - protein, 218 aa, synthetic construct
  CHAIN 1..218: note = Hu29-19
DIVLTQSPDSLAVSLGERATINCRASESVDYYGISSMHWFQQKPGQPPKLLIYRASNLESGIPARFSGSGSRTDFTLTISSLQAEDVAVYYCQQANKDPYTFGGGTKVEIKRTVAAPSVFIFPPSDEQLKSGTASVVCLLNNFYPREAKVQWKVDNALQSGNSQESVTEQDSKDSTYSLSSTLTLSKADYEKHKVYACEVTHQGLSSPVTKSFNRGEC

SEQ ID NO: 42 - protein, 451 aa, synthetic construct
  CHAIN 1..451: note = Hu29-24
QVTLKESGPVLVKPTETLTLTCTVSGFSLTQYAISWVRQPPGKGLEWLGVIWTGGGTNYNSGIKSRLTISKDNSKSQVVLTMTNMDPVDTARYYCVREGDYGSYAGAMDYWGQGTTVTVSSASTKGPSVFPLAPSSKSTSGGTAALGCLVKDYFPEPVTVSWNSGALTSGVHTFPAVLQSSGLYSLSSVVTVPSSSLGTQTYICNVNHKPSNTKVDKKVEPKSCDKTHTCPPCPAPEAAGGPSVFLFPPKPKDTLMISRTPEVTCVVVDVSHEDPEVKFNWYVDGVEVHNAKTKPREEQYNSTYRVVSVLTVLHQDWLNGKEYKCKVSNKALPAPIEKTISKAKGQPREPQVYTLPPSRDELTKNQVSLTCLVKGFYPSDIAVEWESNGQPENNYKTTPPVLDSDGSFFLYSKLTVDKSRWQQGNVFSCSVMHEALHNHYTQKSLSLSPGK

SEQ ID NO: 43 - protein, 218 aa, synthetic construct
  CHAIN 1..218: note = Hu29-24
DIVLTQSPDSLAVSLGQRATINCRASESVDYYGISSMHWFQQKPGQPPKLLIYRASNLESGIPARFSGSGSRTDFTLTISSLQAEDVAVYYCQQANKDPYTFGGGTKVEIKRTVAAPSVFIFPPSDEQLKSGTASVVCLLNNFYPREAKVQWKVDNALQSGNSQESVTEQDSKDSTYSLSSTLTLSKADYEKHKVYACEVTHQGLSSPVTKSFNRGEC

SEQ ID NO: 44 - protein, 444 aa, synthetic construct
  CHAIN 1..444: note = Hu38-4
EFQLVQSGAEVKKPGASVKVSCKASGYTFTDHNMNWVRQAPGQRLEWMGVINPNYGTTTYNQKFKGRVTITVDTSASTAYMELSSLRSEDTAVYYCARRGFAYWGQGTLVTVSSASTKGPSVFPLAPSSKSTSGGTAALGCLVKDYFPEPVTVSWNSGALTSGVHTFPAVLQSSGLYSLSSVVTVPSSSLGTQTYICNVNHKPSNTKVDKKVEPKSCDKTHTCPPCPAPEAAGGPSVFLFPPKPKDTLMISRTPEVTCVVVDVSHEDPEVKFNWYVDGVEVHNAKTKPREEQYNSTYRVVSVLTVLHQDWLNGKEYKCKVSNKALPAPIEKTISKAKGQPREPQVYTLPPSRDELTKNQVSLTCLVKGFYPSDIAVEWESNGQPENNYKTTPPVLDSDGSFFLYSKLTVDKSRWQQGNVFSCSVMHEALHNHYTQKSLSLSPGK

SEQ ID NO: 45 - protein, 219 aa, synthetic construct
  CHAIN 1..219: note = Hu38-4
DIVMTQTPLSLPVTPGEPASISCRSSKSLLYKDGKTYLNWFLQKPGQSPQLLIYLMQTRASGVPDRFSGSGSGTDLTLKISRVEAEDVGVYYCQQIAEYPFTFGSGTKLEIKRTVAAPSVFIFPPSDEQLKSGTASVVCLLNNFYPREAKVQWKVDNALQSGNSQESVTEQDSKDSTYSLSSTLTLSKADYEKHKVYACEVTHQGLSSPVTKSFNRGEC

SEQ ID NO: 46 - protein, 547 aa, synthetic construct
  CHAIN 1..547: note = Hu29-19T
STSCREEQGEFYDHLLRDCISCASICGQHPKQCAAFCEGGGGSGGGGSGGGGSQVTLKESGPVLVKPTETLTLTCTVSGFSLTNYAISWVRQPPGKGLEWLGVIWTGGGTNYNSGIKSRLTISKDNSKSQVVLTMTNMDPVDTARYYCVREGDYGSYAGAMDYWGQGTTVTVSSASTKGPSVFPLAPSSKSTSGGTAALGCLVKDYFPEPVTVSWNSGALTSGVHTFPAVLQSSGLYSLSSVVTVPSSSLGTQTYICNVNHKPSNTKVDKKVEPKSCDKTHTCPPCPAPEAAGGPSVFLFPPKPKDTLMISRTPEVTCVVVDVSHEDPEVKFNWYVDGVEVHNAKTKPREEQYNSTYRVVSVLTVLHQDWLNGKEYKCKVSNKALPAPIEKTISKAKGQPREPQVYTLPPSRDELTKNQVSLTCLVKGFYPSDIAVEWESNGQPENNYKTTPPVLDSDGSFFLYSKLTVDKSRWQQGNVFSCSVMHEALHNHYTQKSLSLSPGGGGSSTSCREEQGEFYDHLLRDCISCASICGQHPKQCAAFCESS

SEQ ID NO: 47 - protein, 547 aa, synthetic construct
  CHAIN 1..547: note = Hu29-24T
STSCREEQGEFYDHLLRDCISCASICGQHPKQCAAFCEGGGGSGGGGSGGGGSQVTLKESGPVLVKPTETLTLTCTVSGFSLTQYAISWVRQPPGKGLEWLGVIWTGGGTNYNSGIKSRLTISKDNSKSQVVLTMTNMDPVDTARYYCVREGDYGSYAGAMDYWGQGTTVTVSSASTKGPSVFPLAPSSKSTSGGTAALGCLVKDYFPEPVTVSWNSGALTSGVHTFPAVLQSSGLYSLSSVVTVPSSSLGTQTYICNVNHKPSNTKVDKKVEPKSCDKTHTCPPCPAPEAAGGPSVFLFPPKPKDTLMISRTPEVTCVVVDVSHEDPEVKFNWYVDGVEVHNAKTKPREEQYNSTYRVVSVLTVLHQDWLNGKEYKCKVSNKALPAPIEKTISKAKGQPREPQVYTLPPSRDELTKNQVSLTCLVKGFYPSDIAVEWESNGQPENNYKTTPPVLDSDGSFFLYSKLTVDKSRWQQGNVFSCSVMHEALHNHYTQKSLSLSPGGGGSSTSCREEQGEFYDHLLRDCISCASICGQHPKQCAAFCESS

SEQ ID NO: 48 - protein, 449 aa, synthetic construct
  CHAIN 1..449: note = Risankizumab
QVQLVQSGAEVKKPGSSVKVSCKASGYTFTDQTIHWMRQAPGQGLEWIGYIYPRDDSPKYNENFKGKVTITADKSTSTAYMELSSLRSEDTAVYYCAIPDRSGYAWFIYWGQGTLVTVSSASTKGPSVFPLAPSSKSTSGGTAALGCLVKDYFPEPVTVSWNSGALTSGVHTFPAVLQSSGLYSLSSVVTVPSSSLGTQTYICNVNHKPSNTKVDKRVEPKSCDKTHTCPPCPAPEAAGGPSVFLFPPKPKDTLMISRTPEVTCVVVDVSHEDPEVKFNWYVDGVEVHNAKTKPREEQYNSTYRVVSVLTVLHQDWLNGKEYKCKVSNKALPAPIEKTISKAKGQPREPQVYTLPPSREEMTKNQVSLTCLVKGFYPSDIAVEWESNGQPENNYKTTPPVLDSDGSFFLYSKLTVDKSRWQQGNVFSCSVMHEALHNHYTQKSLSLSPG

SEQ ID NO: 49 - protein, 214 aa, synthetic construct
  DOMAIN 1..214: note = Risankizumab
DIQMTQSPSSLSASVGDRVTITCKASRDVAIAVAWYQQKPGKVPKLLIYWASTRHTGVPSRFSGSGSRTDFTLTISSLQPEDVADYFCHQYSSYPFTFGSGTKLEIKRTVAAPSVFIFPPSDEQLKSGTASVVCLLNNFYPREAKVQWKVDNALQSGNSQESVTEQDSKDSTYSLSSTLTLSKADYEKHKVYACEVTHQGLSSPVTKSFNRGEC

SEQ ID NO: 50 - protein, 333 aa, synthetic construct
  DOMAIN 1..333: note = RCT-18
SRVDQEERFPQGLWTGVAMRSCPEEQYWDPLLGTCMSCKTICNHQSQRTCAAFCRSLSCRKEQGKFYDHLLRDCISCASICGQHPKQCAYFCENKLRSPVNLPPELDKTHTCPPCPAPEAEGAPSVFLFPPKPKDTLMISRTPEVTCVVVDVSHEDPEVKFNWYVDGVEVHNAKTKPREEQYNSTYRVVSVLTVLHQDWLNGKEYKCKVSNKALPSSIEKTISKAKGQPREPQVYTLPPSRDELTKNQVSLTCLVKGFYPSDIAVEWESNGQPENNYKTTPPVLDSDGSFFLYSKLTVDKSRWQQGNVFSCSVMHEALHNHYTQKSLSLSPGK

SEQ ID NO: 51 - protein, 165 aa, synthetic construct
  DOMAIN 1..165: note = TACI-0
MSGLGRSRRGGRSRVDQEERFPQGLWTGVAMRSCPEEQYWDPLLGTCMSCKTICNHQSQRTCAAFCRSLSCRKEQGKFYDHLLRDCISCASICGQHPKQCAYFCENKLRSPVNLPPELRRQRSGEVENNSDNSGRYQGLEHRGSEASPALPGLKLSADQVALVYS

SEQ ID NO: 52 - protein, 164 aa, synthetic construct
  DOMAIN 1..164: note = TACI-1
SGLGRSRKGGKSRVDQEERFPQGLWTGVAMRSCPEEQYWDPLLGTCMSCKTICNHQSQRTCAAFCRSLSCRKEQGKFYDHLLRDCISCASICGQHPKQCAYFCENKLRSPVNLPPELRKQRSGEVEQNSDNSGKYQGLEHRGSEASPALPGLKLSADQVALVYS

SEQ ID NO: 53 - protein, 133 aa, synthetic construct
  DOMAIN 1..133: note = TACI-2
SGLGRSRKGGKSRVDQEERFPQGLWTGVAMRSCPEEQYWDPLLGTCMSCKTICNHQSQRTCAAFCRSLSCRKEQGKFYDHLLRDCISCASICGQHPKQCAYFCENKLRSPVNLPPELRKQRSGEVENNSDNSG

SEQ ID NO: 54 - protein, 126 aa, synthetic construct
  DOMAIN 1..126: note = TACI-3
SGLGRSRKGGKSRVDQEERFPQGLWTGVAMRSCPEEQYWDPLLGTCMSCKTICNHQSQRTCAAFCRSLSCRKEQGKFYDHLLRDCISCASICGQHPKQCAYFCENKLRSPVNLPPELRKQRSGEVE

SEQ ID NO: 55 - protein, 156 aa, synthetic construct
  DOMAIN 1..156: note = TACI-4
GGRSRVDQEERFPQGLWTGVAMRSCPEEQYWDPLLGTCMSCKTICNHQSQRTCAAFCRSLSCRKEQGKFYDHLLRDCISCASICGQHPKQCAYFCENKLRSPVNLPPELRKQRSGEVENNSDNSGKYQGLEHRGSEASPALPGLKLSADQVALVYS

SEQ ID NO: 56 - protein, 125 aa, synthetic construct
  DOMAIN 1..125: note = TACI-5
GGRSRVDQEERFPQGLWTGVAMRSCPEEQYWDPLLGTCMSCKTICNHQSQRTCAAFCRSLSCRKEQGKFYDHLLRDCISCASICGQHPKQCAYFCENKLRSPVNLPPELRKQRSGEVENNSDNSG

SEQ ID NO: 57 - protein, 118 aa, synthetic construct
  DOMAIN 1..118: note = TACI-6
GGRSRVDQEERFPQGLWTGVAMRSCPEEQYWDPLLGTCMSCKTICNHQSQRTCAAFCRSLSCRKEQGKFYDHLLRDCISCASICGQHPKQCAYFCENKLRSPVNLPPELRKQRSGEVE

SEQ ID NO: 58 - protein, 96 aa, synthetic construct
  DOMAIN 1..96: note = TACI-7
FPQGLWTGVAMRSCPEEQYWDPLLGTCMSCKTICNHQSQRTCAAFCRSLSCRKEQGKFYDHLLRDCISCASICGQHPKQCAYFCENKLRSPVNLPP

SEQ ID NO: 59 - protein, 98 aa, synthetic construct
  DOMAIN 1..98: note = TACI-8
SLSCRKEQGKFYDHLLRDCISCASICGQHPKQCAYFCENKLRSPVNLPPELRKQRSGEVENNSDNSGKYQGLEHRGSEASPALPGLKLSADQVALVYS

SEQ ID NO: 60 - protein, 41 aa, synthetic construct
  DOMAIN 1..41: note = TACI-9
SLSCRKEQGKFYDHLLRDCISCASICGQHPKQCAYFCENKL

SEQ ID NO: 61 - protein, 40 aa, synthetic construct
  DOMAIN 1..40: note = TACI-10
SLSCRKEQGKFYDHLLRDCISCASICGQHPKQCAYFCENK

SEQ ID NO: 62 - protein, 39 aa, synthetic construct
  DOMAIN 1..39: note = TACI-11
SLSCRKEQGKFYDHLLRDCISCASICGQHPKQCAYFCEN

SEQ ID NO: 63 - protein, 38 aa, synthetic construct
  DOMAIN 1..38: note = TACI-12
SLSCRKEQGKFYDHLLRDCISCASICGQHPKQCAYFCE

SEQ ID NO: 64 - protein, 37 aa, synthetic construct
  DOMAIN 1..37: note = TACI-13
SLSCRKEQGKFYDHLLRDCISCASICGQHPKQCAYFC

SEQ ID NO: 65 - protein, 36 aa, synthetic construct
  DOMAIN 1..36: note = TACI-14
SLSCRKEQGKFYDHLLRDCISCASICGQHPKQCAYF

SEQ ID NO: 66 - protein, 41 aa, synthetic construct
  DOMAIN 1..41: note = TACI-9-1
STSCRKEQGKFYDHLLRDCISCASICGQHPKQCAYFCENKL

SEQ ID NO: 67 - protein, 41 aa, synthetic construct
  DOMAIN 1..41: note = TACI-9-2
SLSCSKEQGKFYDHLLRDCISCASICGQHPKQCAYFCENKL

SEQ ID NO: 68 - protein, 41 aa, synthetic construct
  DOMAIN 1..41: note = TACI-9-3
SLSCREEQGKFYDHLLRDCISCASICGQHPKQCAYFCENKL

SEQ ID NO: 69 - protein, 41 aa, synthetic construct
  DOMAIN 1..41: note = TACI-9-4
SLSCRQEQGKFYDHLLRDCISCASICGQHPKQCAYFCENKL

SEQ ID NO: 70 - protein, 41 aa, synthetic construct
  DOMAIN 1..41: note = TACI-9-5
SLSCRKEQGEFYDHLLRDCISCASICGQHPKQCAYFCENKL

SEQ ID NO: 71 - protein, 41 aa, synthetic construct
  DOMAIN 1..41: note = TACI-9-6
SRSCRKEQGKFYDHLLRTCISCASICGQHPKQCAYFCENKL

SEQ ID NO: 72 - protein, 41 aa, synthetic construct
  DOMAIN 1..41: note = TACI-9-7
SRSCRKEQGKFYDHLLRACISCASICGQHPKQCAYFCENKL

SEQ ID NO: 73 - protein, 41 aa, synthetic construct
  DOMAIN 1..41: note = TACI-9-8
SLSCRKEQGKFYDHLLRDCISCASICGQHPKQCAAFCENKL

SEQ ID NO: 74 - protein, 41 aa, synthetic construct
  DOMAIN 1..41: note = TACI-9-9
SRSCRKEQGKFYDHLLRTCISCASICGQHPKQCARFCENKL

SEQ ID NO: 75 - protein, 41 aa, synthetic construct
  DOMAIN 1..41: note = TACI-9-10
SLSCREEQGEFYDHLLRDCISCASICGQHPKQCAYFCENKL

SEQ ID NO: 76 - protein, 41 aa, synthetic construct
  DOMAIN 1..41: note = TACI-9-11
SLSCSEEQGEFYDHLLRDCISCASICGQHPKQCAYFCENKL

SEQ ID NO: 77 - protein, 41 aa, synthetic construct
  DOMAIN 1..41: note = TACI-9-12
STSCRKEQGKFYDHLLRDCISCASICGQHPKQCAAFCENKL

SEQ ID NO: 78 - protein, 41 aa, synthetic construct
  DOMAIN 1..41: note = TACI-9-13
STSCRKEQGKFYDHLLRDCISCASICGQHPKQCAYYCENKL

SEQ ID NO: 79 - protein, 41 aa, synthetic construct
  DOMAIN 1..41: note = TACI-9-14
STSCRKEQGKFYDHLLRDCISCASICGQHPKQCAAYCENKL

SEQ ID NO: 80 - protein, 41 aa, synthetic construct
  DOMAIN 1..41: note = TACI-9-15
STSCREEQGEFYDHLLRDCISCASICGQHPKQCAAFCENKL

SEQ ID NO: 81 - protein, 40 aa, synthetic construct
  DOMAIN 1..40: note = TACI-9-15a
STSCREEQGEFYDHLLRDCISCASICGQHPKQCAAFCENK

SEQ ID NO: 82 - protein, 39 aa, synthetic construct
  DOMAIN 1..39: note = TACI-9-15b
STSCREEQGEFYDHLLRDCISCASICGQHPKQCAAFCEN

SEQ ID NO: 83 - protein, 38 aa, synthetic construct
  DOMAIN 1..38: note = TACI-9-15c
STSCREEQGEFYDHLLRDCISCASICGQHPKQCAAFCE

SEQ ID NO: 84 - protein, 15 aa, synthetic construct
  DOMAIN 1..15: note = 1
GGGGSGGGGSGGGGS

SEQ ID NO: 85 - protein, 4 aa, synthetic construct
  DOMAIN 1..4: note = 2
GGGS